European Patent Application EP 4 588 932 A2, published July 23, 2025. Title: PREPARATION OF FACTOR XA DERIVATIVES. Applicant: Alexion Pharmaceuticals, Inc. The sequence listing filed with the application follows.

SEQUENCE LISTING (11 sequences)

SEQ ID NO: 1 - protein, 448 aa, Homo sapiens [sequence omitted]

SEQ ID NO: 2 - protein, 365 aa, synthetic construct
  REGION 1..365: note = Description of Artificial Sequence: Synthetic polypeptide
ANSFLFWNKYKDGDQCETSPCQNQGKCKDGLGEYTCTCLEGFEGKNCELFTRKLCSLDNGDCDQFCHEEQNSVVCSCARGYTLADNGKACIPTGPYPCGKQTLERRKRRKRIVGGQECKDGECPWQALLINEENEGFCGGTILSEFYILTAAHCLYQAKRFKVRVGDRNTEQEEGGEAVHEVEVVIKHNRFTKETYDFDIAVLRLKTPITFRMNVAPACLPERDWAESTLMTQKTGIVSGFGRTHEKGRQSTRLKMLEVPYVDRNSCKLSSSFIITQNMFCAGYDTKQEDACQGDAGGPHVTRFKDTYFVTGIVSWGEGCARKGKYGIYTKVTAFLKWIDRSMKTRGLPKAKSHAPEVITSSPLK

SEQ ID NO: 3 - protein, 359 aa, synthetic construct
  REGION 1..359: note = Description of Artificial Sequence: Synthetic polypeptide
ANSFLFWNKYKDGDQCETSPCQNQGKCKDGLGEYTCTCLEGFEGKNCELFTRKLCSLDNGDCDQFCHEEQNSVVCSCARGYTLADNGKACIPTGPYPCGKQTLERIVGGQECKDGECPWQALLINEENEGFCGGTILSEFYILTAAHCLYQAKRFKVRVGDRNTEQEEGGEAVHEVEVVIKHNRFTKETYDFDIAVLRLKTPITFRMNVAPACLPERDWAESTLMTQKTGIVSGFGRTHEKGRQSTRLKMLEVPYVDRNSCKLSSSFIITQNMFCAGYDTKQEDACQGDAGGPHVTRFKDTYFVTGIVSWGEGCARKGKYGIYTKVTAFLKWIDRSMKTRGLPKAKSHAPEVITSSPLK

SEQ ID NO: 4 - protein, 105 aa, synthetic construct
  REGION 1..105: note = Description of Artificial Sequence: Synthetic polypeptide
ANSFLFWNKYKDGDQCETSPCQNQGKCKDGLGEYTCTCLEGFEGKNCELFTRKLCSLDNGDCDQFCHEEQNSVVCSCARGYTLADNGKACIPTGPYPCGKQTLER

SEQ ID NO: 5 - protein, 254 aa, synthetic construct
  REGION 1..254: note = Description of Artificial Sequence: Synthetic polypeptide
IVGGQECKDGECPWQALLINEENEGFCGGTILSEFYILTAAHCLYQAKRFKVRVGDRNTEQEEGGEAVHEVEVVIKHNRFTKETYDFDIAVLRLKTPITFRMNVAPACLPERDWAESTLMTQKTGIVSGFGRTHEKGRQSTRLKMLEVPYVDRNSCKLSSSFIITQNMFCAGYDTKQEDACQGDAGGPHVTRFKDTYFVTGIVSWGEGCARKGKYGIYTKVTAFLKWIDRSMKTRGLPKAKSHAPEVITSSPLK

SEQ ID NO: 6 - protein, 6 aa, synthetic construct
  REGION 1..6: note = Description of Artificial Sequence: Synthetic peptide
RKRRKR

SEQ ID NO: 7 - DNA, 1218 bp, synthetic construct
  misc_feature 1..1218: note = Description of Artificial Sequence: Synthetic polynucleotide
  source 1..1218: mol_type = other DNA
atggggcgcccactgcacctcgtcctgctcagtgcctccctggctggcctcctgctgctcggggaaagtctgttcatccgcagggagcaggccaacaacatcctggcgagggtcacgagggccaattcctttcttttctggaataaatacaaagatggcgaccagtgtgagaccagtccttgccagaaccagggcaaatgtaaagacggcctcggggaatacacctgcacctgtttagaaggattcgaaggcaaaaactgtgaattattcacacggaagctctgcagcctggacaacggggactgtgaccagttctgccacgaggaacagaactctgtggtgtgctcctgcgcccgcgggtacaccctggctgacaacggcaaggcctgcattcccacagggccctacccctgtgggaaacagaccctggaacgcaggaagaggaggaagaggatcgtgggaggccaggaatgcaaggacggggagtgtccctggcaggccctgctcatcaatgaggaaaacgagggtttctgtggtggaaccattctgagcgagttctacatcctaacggcagcccactgtctctaccaagccaagagattcaaggtgagggtaggggaccggaacacggagcaggaggagggcggtgaggcggtgcacgaggtggaggtggtcatcaagcacaaccggttcacaaaggagacctatgacttcgacatcgccgtgctccggctcaagacccccatcaccttccgcatgaacgtggcgcctgcctgcctccccgagcgtgactgggccgagtccacgctgatgacgcagaagacggggattgtgagcggcttcgggcgcacccacgagaagggccggcagtccaccaggctcaagatgctggaggtgccctacgtggaccgcaacagctgcaagctgtccagcagcttcatcatcacccagaacatgttctgtgccggctacgacaccaagcaggaggatgcctgccagggggacgcagggggcccgcacgtcacccgcttcaaggacacctacttcgtgacaggcatcgtcagctggggagagggctgtgcccgtaaggggaagtacgggatctacaccaaggtcaccgccttcctcaagtggatcgacaggtccatgaaaaccaggggcttgcccaaggccaagagccatgccccggaggtcataacgtcctctccattaaagtga

SEQ ID NO: 8 - protein, 253 aa, synthetic construct
  REGION 1..253: note = Description of Artificial Sequence: Synthetic polypeptide
IVGGQECKDGECPWQALLINEENEGFCGGTILSEFYILTAAHCLYQAKRFKVRVGDRNTEQEEGGEAVHEVEVVIKHNRFTKETYDFDIAVLRLKTPITFRMNVAPACLPERDWAESTLMTQKTGIVSGFGRTHEKGRQSTRLKMLEVPYVDRNSCKLSSSFIITQNMFCAGYDTKQEDACQGDAGGPHVTRFKDTYFVTGIVSWGEGCARKGKYGIYTKVTAFLKWIDRSMKTRGLPKAKSHAPEVITSSPL

SEQ ID NO: 9 - protein, 241 aa, synthetic construct
  REGION 1..241: note = Description of Artificial Sequence: Synthetic polypeptide
IVGGQECKDGECPWQALLINEENEGFCGGTILSEFYILTAAHCLYQAKRFKVRVGDRNTEQEEGGEAVHEVEVVIKHNRFTKETYDFDIAVLRLKTPITFRMNVAPACLPERDWAESTLMTQKTGIVSGFGRTHEKGRQSTRLKMLEVPYVDRNSCKLSSSFIITQNMFCAGYDTKQEDACQGDAGGPHVTRFKDTYFVTGIVSWGEGCARKGKYGIYTKVTAFLKWIDRSMKTRGLPKAK

SEQ ID NO: 10 - protein, 240 aa, synthetic construct
  REGION 1..240: note = Description of Artificial Sequence: Synthetic polypeptide
IVGGQECKDGECPWQALLINEENEGFCGGTILSEFYILTAAHCLYQAKRFKVRVGDRNTEQEEGGEAVHEVEVVIKHNRFTKETYDFDIAVLRLKTPITFRMNVAPACLPERDWAESTLMTQKTGIVSGFGRTHEKGRQSTRLKMLEVPYVDRNSCKLSSSFIITQNMFCAGYDTKQEDACQGDAGGPHVTRFKDTYFVTGIVSWGEGCARKGKYGIYTKVTAFLKWIDRSMKTRGLPKA

SEQ ID NO: 11 - protein, 239 aa, synthetic construct
  REGION 1..239: note = Description of Artificial Sequence: Synthetic polypeptide
IVGGQECKDGECPWQALLINEENEGFCGGTILSEFYILTAAHCLYQAKRFKVRVGDRNTEQEEGGEAVHEVEVVIKHNRFTKETYDFDIAVLRLKTPITFRMNVAPACLPERDWAESTLMTQKTGIVSGFGRTHEKGRQSTRLKMLEVPYVDRNSCKLSSSFIITQNMFCAGYDTKQEDACQGDAGGPHVTRFKDTYFVTGIVSWGEGCARKGKYGIYTKVTAFLKWIDRSMKTRGLPK